European Patent Specification EP 3 794 142 B1, published July 1, 2026. Title: METHOD. Applicant: OXFORD NANOPORE TECHNOLOGIES LIMITED. The sequence listing filed with the application follows.

SEQUENCE LISTING (11 sequences)

SEQ ID NO: 1 - DNA, 47 bp, Artificial Sequence
  Adaptor Top Strand
gcgtactttttagtacgcttttcggcgtctgcttgggtgtttaacct

SEQ ID NO: 2 - DNA, 47 bp, Artificial Sequence
  Adaptor Top Strand
  misc_feature (1)..(1): deoxyinosine
  misc_feature (2)..(2): deoxyzebularine
  misc_feature (3)..(3): deoxyinosine
  misc_feature (6)..(6): deoxyzebularine
  misc_feature (13)..(13): deoxyinosine
  misc_feature (16)..(16): deoxyzebularine
  misc_feature (17)..(17): deoxyinosine
  misc_feature (18)..(18): deoxyzebularine
nnntantttttantannnttttcggcgtctgcttgggtgtttaacct

SEQ ID NO: 3 - DNA, 24 bp, Artificial Sequence
  Adaptor Bottom Strand
ggttaaacacccaagcagacgccg

SEQ ID NO: 4 - DNA, 22 bp, Artificial Sequence
  Tail for PCR Primer
  misc_feature (1)..(1): deoxyinosine
  misc_feature (2)..(2): deoxyzebularine
  misc_feature (3)..(3): deoxyinosine
  misc_feature (6)..(6): deoxyzebularine
  misc_feature (13)..(13): deoxyinosine
  misc_feature (16)..(16): deoxyzebularine
  misc_feature (17)..(17): deoxyinosine
  misc_feature (18)..(18): deoxyzebularine
nnntantttttantannntttt

SEQ ID NO: 5 - DNA, 70 bp, Artificial Sequence
  Adaptor Top Strand
  modified_base (1)..(1): 5' DBCO-TEG
  misc_feature (17)..(20): C3 Spacer
  misc_feature (21)..(21): deoxyinosine
  misc_feature (22)..(22): deoxyzebularine
  misc_feature (23)..(23): deoxyinosine
  misc_feature (26)..(26): deoxyzebularine
  misc_feature (33)..(33): deoxyinosine
  misc_feature (36)..(36): deoxyzebularine
  misc_feature (37)..(37): deoxyinosine
  misc_feature (38)..(38): deoxyzebularine
gcttgggtgtttaaccnnnnnnntantttttantannnttttgcttacggttcactactcacgacgatgt

SEQ ID NO: 6 - DNA, 70 bp, Artificial Sequence
  Adaptor Top Strand
  modified_base (1)..(1): 5' DBCO-TEG
  misc_feature (17)..(20): C3 Spacer
  misc_feature (21)..(21): deoxyinosine
  misc_feature (22)..(22): deoxyzebularine
  misc_feature (23)..(23): deoxyinosine
  misc_feature (26)..(26): deoxyzebularine
  misc_feature (33)..(33): deoxyinosine
  misc_feature (36)..(36): deoxyzebularine
  misc_feature (37)..(37): deoxyinosine
  misc_feature (38)..(38): deoxyzebularine
gcttgggtgtttaaccnnnnnnntanaaaaatntannnaaaagcttacggttcactactcacgacgatgt

SEQ ID NO: 7 - DNA, 80 bp, Artificial Sequence
  Adaptor Top Strand
  modified_base (1)..(1): 5' DBCO-TEG
  misc_feature (17)..(20): C3 Spacer
  misc_feature (21)..(21): deoxyinosine
  misc_feature (22)..(22): deoxyzebularine
  misc_feature (23)..(23): deoxyinosine
  misc_feature (25)..(25): deoxyzebularine
  misc_feature (26)..(27): deoxyinosine
  misc_feature (31)..(31): deoxyinosine
  misc_feature (38)..(38): deoxyzebularine
  misc_feature (42)..(43): deoxyzebularine
  misc_feature (44)..(44): deoxyinosine
  misc_feature (46)..(46): deoxyzebularine
  misc_feature (47)..(47): deoxyinosine
  misc_feature (48)..(48): deoxyzebularine
gcttgggtgtttaaccnnnnnnnannntatnaaaaatnatannntnnnaaaagcttacggttcactactcacgacgatgt

SEQ ID NO: 8 - DNA, 80 bp, Artificial Sequence
  Adaptor Top Strand
  modified_base (1)..(1): 5' DBCO-TEG
  misc_feature (17)..(20): C3 Spacer
  misc_feature (21)..(21): deoxyzebularine
  misc_feature (23)..(23): deoxyinosine
  misc_feature (26)..(26): deoxyzebularine
  misc_feature (27)..(27): deoxyinosine
  misc_feature (30)..(31): deoxyinosine
  misc_feature (38)..(39): deoxyzebularine
  misc_feature (42)..(42): deoxyzebularine
  misc_feature (43)..(43): deoxyinosine
  misc_feature (46)..(46): deoxyzebularine
  misc_feature (48)..(48): deoxyinosine
gcttgggtgtttaaccnnnnnantanntannaaaaatnntanntantnaaaagcttacggttcactactcacgacgatgt

SEQ ID NO: 9 - DNA, 27 bp, Artificial Sequence
  Adaptor Bottom Strand
catcgtcgtgactagtgaaccgtaagc

SEQ ID NO: 10 - DNA, 27 bp, Artificial Sequence
  Adaptor Bottom Strand
catcgtcgtgagtagtgaaccgtaagc

SEQ ID NO: 11 - DNA, 49 bp, Artificial Sequence
  Adaptor Top Strand
  misc_feature (1)..(1): deoxyinosine
  misc_feature (2)..(2): deoxyzebularine
  misc_feature (3)..(3): deoxyinosine
  misc_feature (6)..(6): deoxyzebularine
  misc_feature (13)..(13): deoxyinosine
  misc_feature (16)..(16): deoxyzebularine
  misc_feature (17)..(17): deoxyinosine
  misc_feature (18)..(18): deoxyzebularine
nnntantttttantannntttgcttacggttcactactcacgacgatgt